European Patent Specification EP 4 039 251 B1, published July 10, 2024. Title: Nanosystems as selective vehicles. Applicant: FUNDACIÓN PARA A INVESTIGACIÓN, DESENVOLVEMENTO E INNOVACIÓN RAMÓN DOMÍNGUEZ. Application EP18382012.5. The sequence listing filed with the application follows.

SEQUENCE LISTING (11 sequences)

SEQ ID NO: 1 - protein, 16 aa, Artificial Sequence
  MOD_RES 1: C18-PEG12
  UROG
NDDCELCVNVACTGCL

SEQ ID NO: 2 - protein, 22 aa, Artificial Sequence
  UROGLys
  DISULFID 10: Disulfide between C in position 10 and 18
  DISULFID 13: disulfide bond between Cys in position 13 and 21
  DISULFID 18: Disulfide between C in position 10 and 18
  DISULFID 22: disulfide bond between Cys in position 13 and 21
KKKKKKNDDCELCVNVACTGCL

SEQ ID NO: 3 - protein, 7 aa, Artificial Sequence
  BRA
CFYDEKR

SEQ ID NO: 4 - protein, 9 aa, Artificial Sequence
  MOD_RES 1: C18-PEG
  RPM
CPIEDRPMC

SEQ ID NO: 5 - protein, 9 aa, Artificial Sequence
  RPM peptide
CPIEDRPMC

SEQ ID NO: 6 - protein, 8 aa, Artificial Sequence
  RPM
VSMSTRPM

SEQ ID NO: 7 - protein, 7 aa, Artificial Sequence
  Control
VSMSTSH

SEQ ID NO: 8 - protein, 8 aa, Artificial Sequence
  RPM-miRNA
  MOD_RES 8: miRNA
VSMSTRPM

SEQ ID NO: 9 - protein, 7 aa, Artificial Sequence
  Control-miRNA
  MOD_RES 7: miRNA
VSMSTSH

SEQ ID NO: 10 - protein, 5 aa, Artificial Sequence
  MOD_RES 1: C18-PEG8
  LAPI
LDFIK

SEQ ID NO: 11 - RNA, 23 nt, Artificial Sequence
  Nucleotide
guccaguuuucccaggaaucccu